European Patent Specification EP 3 375 284 B1, published March 29, 2023. Title: Humanized M-CSF Mice. Applicant: REGENERON PHARMACEUTICALS, INC. YALE UNIVERSITY INSTITUTE FOR RESEARCH IN BIOMEDICINE (IRB). Application 12746594.6. The sequence listing filed with the application follows.

SEQUENCE LISTING (24 sequences)

SEQ ID NO: 1 - DNA, 22 bp, Artificial Sequence
  synthetic oligonucleotide
tactgtagccacatgattggga

SEQ ID NO: 2 - DNA, 20 bp, Artificial Sequence
  synthetic oligonucleotide
cctgtgtcagtcaaaggaac

SEQ ID NO: 3 - DNA, 18 bp, Artificial Sequence
  synthetic oligonucleotide
cgacatggctgggctccc

SEQ ID NO: 4 - DNA, 20 bp, Artificial Sequence
  synthetic oligonucleotide
cgcatggtctcatctattat

SEQ ID NO: 5 - DNA, 27 bp, Artificial Sequence
  synthetic oligonucleotide
gtactgcagaatctctcctttctcctg

SEQ ID NO: 6 - DNA, 30 bp, Artificial Sequence
  synthetic oligonucleotide
gtgtctagatctgacaacctcccaggcaca

SEQ ID NO: 7 - DNA, 20 bp, Artificial Sequence
  synthetic oligonucleotide
ttgtgcttctccactacagc

SEQ ID NO: 8 - DNA, 20 bp, Artificial Sequence
  synthetic oligonucleotide
ctgtaagtctgttaatgaag

SEQ ID NO: 9 - DNA, 24 bp, Artificial Sequence
  synthetic oligonucleotide
aaggacctctcgaagtgttggata

SEQ ID NO: 10 - DNA, 25 bp, Artificial Sequence
  synthetic oligonucleotide
catttaaaaggaactgttgacaacg

SEQ ID NO: 11 - DNA, 20 bp, Artificial Sequence
  synthetic oligonucleotide
cttcctcctcctgaggagtc

SEQ ID NO: 12 - DNA, 20 bp, Artificial Sequence
  synthetic oligonucleotide
cctgaccaaggaaagcaaag

SEQ ID NO: 13 - DNA, 23 bp, Artificial Sequence
  synthetic oligonucleotide
ccaggaatgtccactatggattc

SEQ ID NO: 14 - DNA, 27 bp, Artificial Sequence
  synthetic oligonucleotide
actgctccttgaccctgctctgactca

SEQ ID NO: 15 - DNA, 19 bp, Artificial Sequence
  synthetic oligonucleotide
tgggctgacttcccaaagg

SEQ ID NO: 16 - DNA, 25 bp, Artificial Sequence
  synthetic oligonucleotide
ttaggtgctagtaggctggaaagtg

SEQ ID NO: 17 - DNA, 30 bp, Artificial Sequence
  synthetic oligonucleotide
tgcaatcgcagcttctctccttactaggct

SEQ ID NO: 18 - DNA, 28 bp, Artificial Sequence
  synthetic oligonucleotide
aataggaagaacgaacaggtctaatacc

SEQ ID NO: 19 - DNA, 20 bp, Artificial Sequence
  synthetic oligonucleotide
gctgcttgcctgggttagtg

SEQ ID NO: 20 - DNA, 28 bp, Artificial Sequence
  synthetic oligonucleotide
tgcccaggaacatcaaccactgattctg

SEQ ID NO: 21 - DNA, 22 bp, Artificial Sequence
  synthetic oligonucleotide
gagggacagcagacctcagaag

SEQ ID NO: 22 - DNA, 19 bp, Artificial Sequence
  synthetic oligonucleotide
ggtggagaggctattcggc

SEQ ID NO: 23 - DNA, 23 bp, Artificial Sequence
  synthetic oligonucleotide
tgggcacaacagacaatcggctg

SEQ ID NO: 24 - DNA, 17 bp, Artificial Sequence
  synthetic oligonucleotide
gaacacggcggcatcag